European Patent Application EP 4 653 546 A1, published November 26, 2025. Title: 염기 에디터의 염기 교정 능력을 측정하는 세포외 시험법. Applicant: 주식회사 엣진. Application KR. The sequence listing filed with the application follows.

SEQUENCE LISTING (16 sequences)

SEQ ID NO: 1 - protein, 166 aa, artificial
SEVEFSHEYWMRHALTLAKRARDEREVPVGAVLVLNNRVIGEGWNRAIGLHDPTAHAEIMALRQGGLVMQNYRLIDATLYVTFEPCVMCAGAMIHSRIGRVVFGVRNSKRGAAGSLMNVLNYPGMNHRVEITEGILADECAALLCDFYRMPRQVFNAQKKAQSSIN

SEQ ID NO: 2 - protein, 138 aa, Burkholderia cenocepacia
GSYALGPYQISAPQLPAYNGQTVGTFYYVNDAGGLESKVFSSGGPTPYPNYANAGHVEGQSALFMRDNGISEGLVFHNNPEGTCGFCVNMTETLLPENAKMTVVPPEGAIPVKRGATGETKVFTGNSNSPKSPTKGGC

SEQ ID NO: 3 - protein, 44 aa, artificial
GSYALGPYQISAPQLPAYNGQTVGTFYYVNDAGGLESKVFSSGG

SEQ ID NO: 4 - protein, 94 aa, artificial
PTPYPNYANAGHVEGQSALFMRDNGISEGLVFHNNPEGTCGFCVNMTETLLPENAKMTVVPPEGAIPVKRGATGETKVFTGNSNSPKSPTKGGC

SEQ ID NO: 5 - protein, 108 aa, artificial
GSYALGPYQISAPQLPAYNGQTVGTFYYVNDAGGLESKVFSSGGPTPYPNYANAGHVEGQSALFMRDNGISEGLVFHNNPEGTCGFCVNMTETLLPENAKMTVVPPEG

SEQ ID NO: 6 - protein, 30 aa, artificial
AIPVKRGATGETKVFTGNSNSPKSPTKGGC

SEQ ID NO: 7 - protein, 108 aa, artificial
GSYALGPYQISAPQLPAYNGQTVGTFYYVNDAGGLESKVFISGGPTPYPNYVSAGHVEGQSALFMRDNGISEGLVFHNNPKGTCGFCVNMIETLLPENAAMTVVPPEG

SEQ ID NO: 8 - protein, 30 aa, artificial
AIPVKRGATGETKVFIGNSNSPKSPTKGGC

SEQ ID NO: 9 - protein, 911 aa, artificial
MALSRAVCGTSRQLAPVLGYLGSRQKHSLPDYPYDVPDYAGYPYDVPDYAGYPYDVPDYAGIRIQDLRTLGYSQQQQEKIKPKVRSTVAQHHEALVGHGFTHAHIVALSQHPAALGTVAVKYQDMIAALPEATHEAIVGVGKQWSGARALEALLTVAGELRGPPLQLDTGQLLKIAKRGGVTAVEAVHAWRNALTGAPLNLTPDQVVAIASHDGGKQALETVQRLLPVLCQAHGLTPDQVVAIASNGGGKQALETVQRLLPVLCQDHGLTPAQVVAIASNIGGKQALETVQRLLPVLCQDHGLTPDQVVAIASNNGGKQALETVQRLLPVLCQAHGLTPDQVVAIASHDGGKQALETVQRLLPVLCQDHGLTPDQVVAIASHDGGKQALETVQRLLPVLCQAHGLTPAQVVAIASNGGGKQALETVQRLLPVLCQDHGLTPAQVVAIASNIGGKQALETVQRLLPVLCQAHGLTPDQVVAIASNNGGKQALETVQRLLPVLCQAHGLTPAQVVAIASHDGGKQALETVQRLLPVLCQDHGLTPDQVVAIASHDGGKQALETVQRLLPVLCQAHGLTPEQVVAIASNNGGKQALETVQRLLPVLCQAHGLTPAQVVAIASNGGGKQALETVQRLLPVLCQAHGLTPAQVVAIASNGGGKQALETVQRLLPVLCQAHGLTPEQVVAIASNGGGKQALESIVAQLSRPDPALAALLVGSGSYALGPYQISAPQLPAYNGQTVGTFYYVNDAGGLESKVFSSGGPTPYPNYANAGHVEGQSALFMRDNGISEGLVFHNNPEGTCGFCVNMTETLLPENAKMTVVPPEGSGGSTNLSDIIEKETGKQLVIQESILMLPEEVEEVIGNKPESDILVHTAYDESTDENVMLLTSDAPEYKPWALVIQDSNGENKIKML

SEQ ID NO: 10 - protein, 927 aa, artificial
MASVLTPLLLRGLTGSARRLPVPRAKIHSLDYKDHDGDYKDHDIDYKDDDDKGIRIQDLRTLGYSQQQQEKIKPKVRSTVAQHHEALVGHGFTHAHIVALSQHPAALGTVAVKYQDMIAALPEATHEAIVGVGKQWSGARALEALLTVAGELRGPPLQLDTGQLLKIAKRGGVTAVEAVHAWRNALTGAPLNLTPDQVVAIASNNGGKQALETVQRLLPVLCQDHGLTPAQVVAIASNIGGKQALETVQRLLPVLCQAHGLTPEQVVAIASNNGGKQALETVQRLLPVLCQAHGLTPDQVVAIASNGGGKQALETVQRLLPVLCQAHGLTPAQVVAIASNGGGKQALETVQRLLPVLCQAHGLTPEQVVAIASNGGGKQALETVQRLLPVLCQAHGLTPAQVVAIASNNGGKQALETVQRLLPVLCQDHGLTPAQVVAIASNIGGKQALETVQRLLPVLCQAHGLTPEQVVAIASNGGGKQALETVQRLLPVLCQAHGLTPDQVVAIASNNGGKQALETVQRLLPVLCQAHGLTPAQVVAIASHDGGKQALETVQRLLPVLCQDHGLTPDQVVAIASNGGGKQALETVQRLLPVLCQAHGLTPDQVVAIASHDGGKQALETVQRLLPVLCQAHGLTPDQVVAIASNIGGKQALETVQRLLPVLCQAHGLTPAQVVAIASHDGGKQALETVQRLLPVLCQAHGLTPAQVVAIASHDGGKQALETVQRLLPVLCQDHGLTPAQVVAIASHDGGKQALETVQRLLPVLCQAHGLTPEQVVAIASNGGGKQALESIVAQLSRPDPALAALLVGSAIPVKRGATGETKVFTGNSNSPKSPTKGGCSGGSTNLSDIIEKETGKQLVIQESILMLPEEVEEVIGNKPESDILVHTAYDESTDENVMLLTSDAPEYKPWALVIQDSNGENKIKML

SEQ ID NO: 11 - protein, 952 aa, artificial
MALSRAVCGTSRQLAPVLGYLGSRQKHSLPDYPYDVPDYAGYPYDVPDYAGYPYDVPDYAGIRIQDLRTLGYSQQQQEKIKPKVRSTVAQHHEALVGHGFTHAHIVALSQHPAALGTVAVKYQDMIAALPEATHEAIVGVGKQWSGARALEALLTVAGELRGPPLQLDTGQLLKIAKRGGVTAVEAVHAWRNALTGAPLNLTPDQVVAIASHDGGKQALETVQRLLPVLCQAHGLTPDQVVAIASNGGGKQALETVQRLLPVLCQDHGLTPAQVVAIASNIGGKQALETVQRLLPVLCQDHGLTPDQVVAIASNNGGKQALETVQRLLPVLCQAHGLTPDQVVAIASHDGGKQALETVQRLLPVLCQDHGLTPDQVVAIASHDGGKQALETVQRLLPVLCQAHGLTPAQVVAIASNGGGKQALETVQRLLPVLCQDHGLTPAQVVAIASNIGGKQALETVQRLLPVLCQAHGLTPDQVVAIASNNGGKQALETVQRLLPVLCQAHGLTPAQVVAIASHDGGKQALETVQRLLPVLCQDHGLTPDQVVAIASHDGGKQALETVQRLLPVLCQAHGLTPEQVVAIASNNGGKQALETVQRLLPVLCQAHGLTPAQVVAIASNGGGKQALETVQRLLPVLCQAHGLTPAQVVAIASNGGGKQALETVQRLLPVLCQAHGLTPEQVVAIASNGGGKQALESIVAQLSRPDPALAALTNDHLVALACLGGRPALDAVKKGLLVGSAIPVKRGATGETKVFTGNSNSPKSPTKGGCSGSETPGTSESATPESSEVEFSHEYWMRHALTLAKRARDEREVPVGAVLVLNNRVIGEGWNRAIGLHDPTAHAEIMALRQGGLVMQNYRLIDATLYVTFEPCVMCAGAMIHSRIGRVVFGVRNSKRGAAGSLMNVLNYPGMNHRVEITEGILADECAALLCDFYRMPRQVFNAQKKAQSSIN

SEQ ID NO: 12 - protein, 943 aa, artificial
MASVLTPLLLRGLTGSARRLPVPRAKIHSLDYKDHDGDYKDHDIDYKDDDDKGIRIQDLRTLGYSQQQQEKIKPKVRSTVAQHHEALVGHGFTHAHIVALSQHPAALGTVAVKYQDMIAALPEATHEAIVGVGKQWSGARALEALLTVAGELRGPPLQLDTGQLLKIAKRGGVTAVEAVHAWRNALTGAPLNLTPDQVVAIASNNGGKQALETVQRLLPVLCQDHGLTPAQVVAIASNIGGKQALETVQRLLPVLCQAHGLTPEQVVAIASNNGGKQALETVQRLLPVLCQAHGLTPDQVVAIASNGGGKQALETVQRLLPVLCQAHGLTPAQVVAIASNGGGKQALETVQRLLPVLCQAHGLTPEQVVAIASNGGGKQALETVQRLLPVLCQAHGLTPAQVVAIASNNGGKQALETVQRLLPVLCQDHGLTPAQVVAIASNIGGKQALETVQRLLPVLCQAHGLTPEQVVAIASNGGGKQALETVQRLLPVLCQAHGLTPDQVVAIASNNGGKQALETVQRLLPVLCQAHGLTPAQVVAIASHDGGKQALETVQRLLPVLCQDHGLTPDQVVAIASNGGGKQALETVQRLLPVLCQAHGLTPDQVVAIASHDGGKQALETVQRLLPVLCQAHGLTPDQVVAIASNIGGKQALETVQRLLPVLCQAHGLTPAQVVAIASHDGGKQALETVQRLLPVLCQAHGLTPAQVVAIASHDGGKQALETVQRLLPVLCQDHGLTPAQVVAIASHDGGKQALETVQRLLPVLCQAHGLTPEQVVAIASNGGGKQALESIVAQLSRPDPALAALTNDHLVALACLGGRPALDAVKKGLGGSGSGSYALGPYQISAPQLPAYNGQTVGTFYYVNDAGGLESKVFSSGGPTPYPNYANAGHVEGQSALFMRDNGISEGLVFHNNPEGTCGFCVNMTETLLPENAKMTVVPPEG

SEQ ID NO: 13 - protein, 978 aa, artificial
MASVLTPLLLRGLTGSARRLPVPRAKIHSLDYKDHDGDYKDHDIDYKDDDDKGIRIQDLRTLGYSQQQQEKIKPKVRSTVAQHHEALVGHGFTHAHIVALSQHPAALGTVAVKYQDMIAALPEATHEAIVGVGKQWSGARALEALLTVAGELRGPPLQLDTGQLLKIAKRGGVTAVEAVHAWRNALTGAPLNLTPDQVVAIASNIGGKQALETVQRLLPVLCQDHGLTPDQVVAIASHDGGKQALETVQRLLPVLCQAHGLTPAQVVAIASNNGGKQALETVQRLLPVLCQDHGLTPEQVVAIASNNGGKQALETVQRLLPVLCQAHGLTPAQVVAIASNNGGKQALETVQRLLPVLCQDHGLTPDQVVAIASHDGGKQALETVQRLLPVLCQDHGLTPEQVVAIASNGGGKQALETVQRLLPVLCQAHGLTPDQVVAIASNIGGKQALETVQRLLPVLCQAHGLTPAQVVAIASHDGGKQALETVQRLLPVLCQAHGLTPEQVVAIASNGGGKQALETVQRLLPVLCQAHGLTPDQVVAIASNIGGKQALETVQRLLPVLCQAHGLTPAQVVAIASHDGGKQALETVQRLLPVLCQDHGLTPDQVVAIASNIGGKQALETVQRLLPVLCQDHGLTPAQVVAIASNIGGKQALETVQRLLPVLCQAHGLTPAQVVAIASHDGGKQALETVQRLLPVLCQAHGLTPEQVVAIASNGGGKQALESIVAQLSRPDPALAALTNDHLVALACLGGRPALDAVKKGLLVGSAIPVKRGATGETKVFTGNSNSPKSPTKGGCSGSETPGTSESATPESSEVEFSHEYWMRHALTLAKRARDEREVPVGAVLVLNNRVIGEGWNRAIGLHDPTAHAEIMALRQGGLVMQNYRLIDATLYVTFEPCVMCAGAMIHSRIGRVVFGVRNSKRGAAGSLMNVLNYPGMNHRVEITEGILADECAALLCDFYRMPRQVFNAQKKAQSSIN

SEQ ID NO: 14 - protein, 1012 aa, artificial
MASVLTPLLLRGLTGSARRLPVPRAKIHSLDYKDHDGDYKDHDIDYKDDDDKGIRIQDLRTLGYSQQQQEKIKPKVRSTVAQHHEALVGHGFTHAHIVALSQHPAALGTVAVKYQDMIAALPEATHEAIVGVGKQWSGARALEALLTVAGELRGPPLQLDTGQLLKIAKRGGVTAVEAVHAWRNALTGAPLNLTPDQVVAIASNIGGKQALETVQRLLPVLCQDHGLTPDQVVAIASHDGGKQALETVQRLLPVLCQAHGLTPAQVVAIASNNGGKQALETVQRLLPVLCQDHGLTPEQVVAIASNNGGKQALETVQRLLPVLCQAHGLTPAQVVAIASNNGGKQALETVQRLLPVLCQDHGLTPDQVVAIASHDGGKQALETVQRLLPVLCQDHGLTPEQVVAIASNGGGKQALETVQRLLPVLCQAHGLTPDQVVAIASNIGGKQALETVQRLLPVLCQAHGLTPAQVVAIASHDGGKQALETVQRLLPVLCQAHGLTPEQVVAIASNGGGKQALETVQRLLPVLCQAHGLTPDQVVAIASNIGGKQALETVQRLLPVLCQAHGLTPAQVVAIASHDGGKQALETVQRLLPVLCQDHGLTPDQVVAIASNIGGKQALETVQRLLPVLCQDHGLTPAQVVAIASNIGGKQALETVQRLLPVLCQAHGLTPAQVVAIASHDGGKQALETVQRLLPVLCQDHGLTPAQVVAIASHDGGKQALETVQRLLPVLCQAHGLTPEQVVAIASNGGGKQALESIVAQLSRPDPALAALTNDHLVALACLGGRPALDAVKKGLLVGSAIPVKRGATGETKVFTGNSNSPKSPTKGGCSGSETPGTSESATPESSEVEFSHEYWMRHALTLAKRARDEREVPVGAVLVLNNRVIGEGWNRAIGLHDPTAHAEIMALRQGGLVMQNYRLIDATLYVTFEPCVMCAGAMIHSRIGRVVFGVRNSKRGAAGSLMNVLNYPGMNHRVEITEGILADECAALLCDFYRMPRQVFNAQKKAQSSIN

SEQ ID NO: 15 - protein, 849 aa, artificial
MALSRAVCGTSRQLAPVLGYLGSRQKHSLPDYPYDVPDYAGYPYDVPDYAGYPYDVPDYAGIRIQDLRTLGYSQQQQEKIKPKVRSTVAQHHEALVGHGFTHAHIVALSQHPAALGTVAVKYQDMIAALPEATHEAIVGVGKQWSGARALEALLTVAGELRGPPLQLDTGQLLKIAKRGGVTAVEAVHAWRNALTGAPLNLTPAQVVAIASHDGGKQALETVQRLLPVLCQAHGLTPDQVVAIASNGGGKQALETVQRLLPVLCQAHGLTPAQVVAIASNGGGKQALETVQRLLPVLCQDHGLTPEQVVAIASNGGGKQALETVQRLLPVLCQAHGLTPAQVVAIASNNGGKQALETVQRLLPVLCQDHGLTPDQVVAIASNNGGKQALETVQRLLPVLCQDHGLTPAQVVAIASNGGGKQALETVQRLLPVLCQAHGLTPAQVVAIASNNGGKQALETVQRLLPVLCQDHGLTPAQVVAIASNIGGKQALETVQRLLPVLCQAHGLTPDQVVAIASNIGGKQALETVQRLLPVLCQDHGLTPAQVVAIASNNGGKQALETVQRLLPVLCQDHGLTPAQVVAIASNIGGKQALETVQRLLPVLCQAHGLTPDQVVAIASNNGGKQALETVQRLLPVLCQAHGLTPAQVVAIASNGGGKQALETVQRLLPVLCQAHGLTPEQVVAIASNGGGKQALESIVAQLSRPDPALAALTNDHLVALACLGGRPALDAVKKGLGGSGSGSYALGPYQISAPQLPAYNGQTVGTFYYVNDAGGLESKVFSSGGPTPYPNYANAGHVEGQSALFMRDNGISEGLVFHNNPEGTCGFCVNMTETLLPENAKMTVVPPEG

SEQ ID NO: 16 - protein, 883 aa, artificial
MALSRAVCGTSRQLAPVLGYLGSRQKHSLPDYPYDVPDYAGYPYDVPDYAGYPYDVPDYAGIRIQDLRTLGYSQQQQEKIKPKVRSTVAQHHEALVGHGFTHAHIVALSQHPAALGTVAVKYQDMIAALPEATHEAIVGVGKQWSGARALEALLTVAGELRGPPLQLDTGQLLKIAKRGGVTAVEAVHAWRNALTGAPLNLTPAQVVAIASHDGGKQALETVQRLLPVLCQAHGLTPDQVVAIASNGGGKQALETVQRLLPVLCQAHGLTPAQVVAIASNGGGKQALETVQRLLPVLCQDHGLTPEQVVAIASNGGGKQALETVQRLLPVLCQAHGLTPAQVVAIASNNGGKQALETVQRLLPVLCQDHGLTPDQVVAIASNNGGKQALETVQRLLPVLCQDHGLTPAQVVAIASNGGGKQALETVQRLLPVLCQAHGLTPAQVVAIASNNGGKQALETVQRLLPVLCQDHGLTPAQVVAIASNIGGKQALETVQRLLPVLCQAHGLTPDQVVAIASNIGGKQALETVQRLLPVLCQDHGLTPAQVVAIASNNGGKQALETVQRLLPVLCQDHGLTPAQVVAIASNIGGKQALETVQRLLPVLCQAHGLTPDQVVAIASNNGGKQALETVQRLLPVLCQAHGLTPDQVVAIASNGGGKQALETVQRLLPVLCQAHGLTPAQVVAIASNGGGKQALETVQRLLPVLCQAHGLTPEQVVAIASNGGGKQALESIVAQLSRPDPALAALTNDHLVALACLGGRPALDAVKKGLGGSGSGSYALGPYQISAPQLPAYNGQTVGTFYYVNDAGGLESKVFSSGGPTPYPNYANAGHVEGQSALFMRDNGISEGLVFHNNPEGTCGFCVNMTETLLPENAKMTVVPPEG